European Patent Application EP 4 509 608 A1, published February 19, 2025. Title: Capped RNA and method for producing thereof, protein production device and method for producing protein. Applicant: JAPAN SCIENCE AND TECHNOLOGY AGENCY. Application WO. The sequence listing filed with the application follows.

SEQUENCE LISTING (64 sequences)

SEQ ID NO: 1 - RNA, 20 nt, synthetic construct
  misc_feature 1..20: note = RNA1
  misc_feature 1: note = 5' is monophosphate
  source 1..20: mol_type = other RNA
gcgtcaccttaatatgcgcc

SEQ ID NO: 2 - RNA, 21 nt, synthetic construct
  misc_feature 1..21: note = RNA2
  misc_feature 1: note = 5' is monophosphate
  misc_feature 1^2: note = C4 linker
  source 1..21: mol_type = other RNA
ggcgtcaccttaatatgcgcc

SEQ ID NO: 3 - RNA, 20 nt, synthetic construct
  misc_feature 1..20: note = RNA3
  misc_feature 1: note = 5' is monophosphate
  misc_feature 1: note = C4 linker
  source 1..20: mol_type = other RNA
gcgtcaccttaatatgcgcc

SEQ ID NO: 4 - RNA, 20 nt, synthetic construct
  misc_feature 1..20: note = RNA4
  misc_feature 20: note = 3' is monophosphate
  misc_feature 20: note = C4 linker
  source 1..20: mol_type = other RNA
gcgtcaccttaatatgcgcc

SEQ ID NO: 5 - RNA, 20 nt, synthetic construct
  misc_feature 1..20: note = RNA5
  misc_feature 1: note = 5' is monophosphate
  source 1..20: mol_type = other RNA
cgccgtggaactatctccta

SEQ ID NO: 6 - RNA, 50 nt, synthetic construct
  misc_feature 1..50: note = RNA6
  misc_feature 1: note = 5' is monophosphate
  source 1..50: mol_type = other RNA
gcgtcaccttaatatgcgccaaaaaaaaaaaaaaaaaaaaaaaaaaaaaa

SEQ ID NO: 7 - RNA, 51 nt, synthetic construct
  misc_feature 1..51: note = RNA7
  misc_feature 1: note = 5' is monophosphate
  misc_feature 1^2: note = C4 linker
  source 1..51: mol_type = other RNA
ggcgtcaccttaatatgcgccaaaaaaaaaaaaaaaaaaaaaaaaaaaaaa

SEQ ID NO: 8 - RNA, 50 nt, synthetic construct; identical to SEQ ID NO: 6
  misc_feature 1..50: note = RNA8
  misc_feature 1: note = 5' is monophosphate
  misc_feature 1: note = C4 linker
  source 1..50: mol_type = other RNA

SEQ ID NO: 9 - RNA, 50 nt, synthetic construct; identical to SEQ ID NO: 6
  misc_feature 1..50: note = RNA9
  misc_feature 1: note = 5' is monophosphate
  modified_base 1: mod_base = gm
  source 1..50: mol_type = other RNA

SEQ ID NO: 10 - RNA, 50 nt, synthetic construct; identical to SEQ ID NO: 6
  misc_feature 1..50: note = RNA10
  misc_feature 1: note = 5' is monophosphate
  modified_base 1: mod_base = gm
  misc_feature 1: note = C4 linker
  source 1..50: mol_type = other RNA

SEQ ID NO: 11 - RNA, 50 nt, synthetic construct; identical to SEQ ID NO: 6
  misc_feature 1..50: note = RNA11
  misc_feature 1: note = 5' is monophosphate
  misc_feature 1..3: note = LNA
  misc_feature 18..20: note = LNA
  source 1..50: mol_type = other RNA

SEQ ID NO: 12 - RNA, 50 nt, synthetic construct; identical to SEQ ID NO: 6
  misc_feature 1..50: note = RNA12
  misc_feature 1: note = 5' is monophosphate
  misc_feature 1: note = C4 linker
  misc_feature 1..3: note = LNA
  misc_feature 18..20: note = LNA
  source 1..50: mol_type = other RNA

SEQ ID NO: 13 - RNA, 21 nt, synthetic construct
  misc_feature 1..21: note = Capped RNA1 (5' capp probe in Fig.3)
  modified_base 1: mod_base = m7g
  misc_feature 1^2: note = triphosphate linkage
  source 1..21: mol_type = other RNA
ggcgtcaccttaatatgcgcc

SEQ ID NO: 14 - RNA, 21 nt, synthetic construct
  misc_feature 1..21: note = Capped RNA2(5' capp probe in Fig.3)
  modified_base 1: mod_base = m7g
  misc_feature 1^2: note = triphosphate linkage
  misc_feature 2^3: note = C4 linker
  source 1..21: mol_type = other RNA
ggcgtcaccttaatatgcgcc

SEQ ID NO: 15 - RNA, 21 nt, synthetic construct
  misc_feature 1..21: note = Capped RNA3
  modified_base 1: mod_base = m7g
  misc_feature 1^2: note = triphosphate linkage
  misc_feature 1^2: note = C4 linker
  source 1..21: mol_type = other RNA
ggcgtcaccttaatatgcgcc

SEQ ID NO: 16 - RNA, 21 nt, synthetic construct
  misc_feature 1..21: note = Capped RNA4 (3' capp probe in Fig.3)
  misc_feature 20^21: note = triphosphate linkage
  misc_feature 20^21: note = C4 linker
  modified_base 21: mod_base = m7g
  source 1..21: mol_type = other RNA
gcgtcaccttaatatgcgccg

SEQ ID NO: 17 - RNA, 21 nt, synthetic construct
  misc_feature 1..21: note = Capped RNA5
  modified_base 1: mod_base = m7g
  misc_feature 1^2: note = triphosphate linkage
  source 1..21: mol_type = other RNA
gcgccgtggaactatctccta

SEQ ID NO: 18 - RNA, 51 nt, synthetic construct; identical to SEQ ID NO: 7
  misc_feature 1..51: note = Capped RNA6
  modified_base 1: mod_base = m7g
  source 1..51: mol_type = other RNA

SEQ ID NO: 19 - RNA, 52 nt, synthetic construct
  misc_feature 1..52: note = Capped RNA7 (5' capp probe with poly A in Fig.3)
  modified_base 1: mod_base = m7g
  misc_feature 1^2: note = triphosphate linkage
  misc_feature 2^3: note = C4 linker
  source 1..52: mol_type = other RNA
gggcgtcaccttaatatgcgccaaaaaaaaaaaaaaaaaaaaaaaaaaaaaa

SEQ ID NO: 20 - RNA, 51 nt, synthetic construct; identical to SEQ ID NO: 7
  misc_feature 1..51: note = Capped RNA8 (5' capp probe with poly A in Fig.3)
  modified_base 1: mod_base = m7g
  misc_feature 1^2: note = triphosphate linkage
  misc_feature 1^2: note = C4 linker
  source 1..51: mol_type = other RNA

SEQ ID NO: 21 - RNA, 51 nt, synthetic construct; identical to SEQ ID NO: 7
  misc_feature 1..51: note = Capped RNA9
  modified_base 1: mod_base = m7g
  misc_feature 1^2: note = triphosphate linkage
  modified_base 2: mod_base = gm
  source 1..51: mol_type = other RNA

SEQ ID NO: 22 - RNA, 51 nt, synthetic construct; identical to SEQ ID NO: 7
  misc_feature 1..51: note = Capped RNA10
  modified_base 1: mod_base = m7g
  misc_feature 1^2: note = triphosphate linkage
  misc_feature 1^2: note = C4 linker
  modified_base 2: mod_base = gm
  source 1..51: mol_type = other RNA

SEQ ID NO: 23 - RNA, 51 nt, synthetic construct; identical to SEQ ID NO: 7
  misc_feature 1..51: note = Capped RNA11
  modified_base 1: mod_base = m7g
  misc_feature 1^2: note = triphosphate linkage
  misc_feature 2..4: note = LNA
  misc_feature 18..20: note = LNA
  source 1..51: mol_type = other RNA

SEQ ID NO: 24 - RNA, 51 nt, synthetic construct; identical to SEQ ID NO: 7
  misc_feature 1..51: note = Capped RNA12
  modified_base 1: mod_base = m7g
  misc_feature 1^2: note = triphosphate linkage
  misc_feature 1^2: note = C4 linker
  misc_feature 2..4: note = LNA
  misc_feature 18..20: note = LNA
  source 1..51: mol_type = other RNA

SEQ ID NO: 25 - DNA, 48 bp, synthetic construct
  misc_feature 1..48: note = primer_Fw
  source 1..48: mol_type = other DNA
cccggatcctaatacgactcactataggtcttcacactcgaagatttc

SEQ ID NO: 26 - DNA, 51 bp, synthetic construct
  misc_feature 1..51: note = primer_Rev
  source 1..51: mol_type = other DNA
ttttttttttttttttttttttttttttttctagaattacgccagaatgcg

SEQ ID NO: 27 - DNA, 30 bp, synthetic construct
  misc_feature 1..30: note = Splint_1
  source 1..30: mol_type = other DNA
accttaatatgcgccttttttttttttttt

SEQ ID NO: 28 - DNA, 30 bp, synthetic construct
  misc_feature 1..30: note = Splint_2
  source 1..30: mol_type = other DNA
tcgagtgtgaagaccatggtggctttaccc

SEQ ID NO: 29 - RNA, 107 nt, synthetic construct
  misc_feature 1..107: note = blanch RNA
  modified_base 1: mod_base = gm
  misc_feature 1^2: note = The 2'-methylguanosine(Gm) and the adenosine(A) are linked by abranching linker. The number of Gm's correspond to the number ofthe branches of the linker. Cap structure can be introduced tothe each 5' end of the Gm.
  source 1..107: mol_type = other RNA
ggagccaccatggactacaaggacgacgacgataagatcatcgactataaagacgacgacgataaacaccaccaccaccaccactgaaaaaaaaaaaaaaaaaaaaa

SEQ ID NO: 30 - RNA, 50 nt, synthetic construct
  misc_feature 1..50: note = bicistronic mRNA
  source 1..50: mol_type = other RNA
gacagtctgctcgaagcggccgctctagaagcgtcaccttaatatgcgcc

SEQ ID NO: 31 - RNA, 650 nt, synthetic construct
  misc_feature 1..650: note = RNA coding nanoluciferase
  source 1..650: mol_type = other RNA
ggcgcatattaaggtgacgcgtgtggcctcgaacaccgagcgaccctgcagcgacccgcttaaaagcttggcaatccggtactgttggtaaagccaccatggtcttcacactcgaagatttcgttggggactggcgacagacagccggctacaacctggaccaagtccttgaacagggaggtgtgtccagtttgtttcagaatctcggggtgtccgtaactccgatccaaaggattgtcctgagcggtgaaaatgggctgaagatcgacatccatgtcatcatcccgtatgaaggtctgagcggcgaccaaatgggccagatcgaaaaaatttttaaggtggtgtaccctgtggatgatcatcactttaaggtgatcctgcactatggcacactggtaatcgacggggttacgccgaacatgatcgactatttcggacggccgtatgaaggcatcgccgtgttcgacggcaaaaagatcactgtaacagggaccctgtggaacggcaacaaaattatcgacgagcgcctgatcaaccccgacggctccctgctgttccgagtaaccatcaacggagtgaccggctggcggctgtgcgaacgcattctggcgtaattctagaaaaaaaaaaaaaaaaaaaaaaaaaaaaaa

SEQ ID NO: 32 - DNA, 676 bp, synthetic construct
  misc_feature 1..676: note = DNA templete of nanoluciferase coding RNA
  source 1..676: mol_type = other DNA
cccggatcctaatacgactcactataggcgcatattaaggtgacgcgtgtggcctcgaacaccgagcgaccctgcagcgacccgcttaaaagcttggcaatccggtactgttggtaaagccaccatggtcttcacactcgaagatttcgttggggactggcgacagacagccggctacaacctggaccaagtccttgaacagggaggtgtgtccagtttgtttcagaatctcggggtgtccgtaactccgatccaaaggattgtcctgagcggtgaaaatgggctgaagatcgacatccatgtcatcatcccgtatgaaggtctgagcggcgaccaaatgggccagatcgaaaaaatttttaaggtggtgtaccctgtggatgatcatcactttaaggtgatcctgcactatggcacactggtaatcgacggggttacgccgaacatgatcgactatttcggacggccgtatgaaggcatcgccgtgttcgacggcaaaaagatcactgtaacagggaccctgtggaacggcaacaaaattatcgacgagcgcctgatcaaccccgacggctccctgctgttccgagtaaccatcaacggagtgaccggctggcggctgtgcgaacgcattctggcgtaattctagtttttttttttttttttttttttttttttt

SEQ ID NO: 33 - RNA, 54 nt, synthetic construct
  misc_feature 1..54: note = Synthesis of branched RNA-1
  misc_feature 14^15: note = The guanosine(G) and the uridine(U) are linked by a branchinglinker. GmGmAGCG is linked to the branched chain that branchesoff from the main chain. ("Gm" indicates 2'OMe guanosine). A capstructure can be attached to the 5' end of the Gm.
  source 1..54: mol_type = other RNA
ggcgcatattaaggtgacgcgtgtggcctcgaacaccgagggtaaagccaccat

SEQ ID NO: 34 - RNA, 2489 nt, synthetic construct
  misc_feature 1..2489: note = bicistronic RNA coding firefly-luciferase and nano-luciferase
  modified_base 1: mod_base = m7g
  source 1..2489: mol_type = other RNA
gggcgaattcgagcggcattccggtactgttggttttgccaccatggactacaaggacgacgacgacaagatcatcgactataaagacgacgacgataaaggtggcgactataaggacgacgacgacaaagccaccatggaagacgccaaaaacataaagaaaggcccggcgccattctatccgctggaagatggaaccgctggagagcaactgcataaggctatgaagagatacgccctggttcctggaacaattgcttttacagatgcacatatcgaggtggacatcacttacgctgagtacttcgaaatgtccgttcggttggcagaagctatgaaacgatatgggctgaatacaaatcacagaatcgtcgtatgcagtgaaaactctcttcaattctttatgccggtgttgggcgcgttatttatcggagttgcagttgcgcccgcgaacgacatttataatgaacgtgaattgctcaacagtatgggcatttcgcagcctaccgtggtgttcgtttccaaaaaggggttgcaaaaaattttgaacgtgcaaaaaaagctcccaatcatccaaaaaattattatcatggattctaaaacggattaccagggatttcagtcgatgtacacgttcgtcacatctcatctacctcccggttttaatgaatacgattttgtgccagagtccttcgatagggacaagacaattgcactgatcatgaactcctctggatctactggtctgcctaaaggtgtcgctctgcctcatagaactgcctgcgtgagattctcgcatgccagagatcctatttttggcaatcaaatcattccggatactgcgattttaagtgttgttccattccatcacggttttggaatgtttactacactcggatatttgatatgtggatttcgagtcgtcttaatgtatagatttgaagaagagctgtttctgaggagccttcaggattacaagattcaaagtgcgctgctggtgccaaccctattctccttcttcgccaaaagcactctgattgacaaatacgatttatctaatttacacgaaattgcttctggtggcgctcccctctctaaggaagtcggggaagcggttgccaagaggttccatctgccaggtatcaggcaaggatatgggctcactgagactacatcagctattctgattacacccgagggggatgataaaccgggcgcggtcggtaaagttgttccattttttgaagcgaaggttgtggatctggataccgggaaaacgctgggcgttaatcaaagaggcgaactgtgtgtgagaggtcctatgattatgtccggttatgtaaacaatccggaagcgaccaacgccttgattgacaaggatggatggctacattctggagacatagcttactgggacgaagacgaacacttcttcatcgttgaccgcctgaagtctctgattaagtacaaaggctatcaggtggctcccgctgaattggaatccatcttgctccaacaccccaacatcttcgacgcaggtgtcgcaggtcttcccgacgatgacgccggtgaacttcccgccgccgttgttgttttggagcacggaaagacgatgacggaaaaagagatcgtggattacgtcgccagtcaagtaacaaccgcgaaaaagttgcgcggaggagttgtgtttgtggacgaagtaccgaaaggtcttaccggaaaactcgacgcaagaaaaatcagagagatcctcataaaggccaagaagggcggaaagatcgccgtgtaattctagagtcggggcggccggccgcttcgagcagacacgataagatacagggcgcatattaaggtgacgcgtgtggcctcgaacaccgagcgaccctgcagcgacccgcttaaaagcttggcaatccggtactgttggtaaagccaccatggtcttcacactcgaagatttcgttggggactggcgacagacagccggctacaacctggaccaagtccttgaacagggaggtgtgtccagtttgtttcagaatctcggggtgtccgtaactccgatccaaaggattgtcctgagcggtgaaaatgggctgaagatcgacatccatgtcatcatcccgtatgaaggtctgagcggcgaccaaatgggccagatcgaaaaaatttttaaggtggtgtaccctgtggatgatcatcactttaaggtgatcctgcactatggcacactggtaatcgacggggttacgccgaacatgatcgactatttcggacggccgtatgaaggcatcgccgtgttcgacggcaaaaagatcactgtaacagggaccctgtggaacggcaacaaaattatcgacgagcgcctgatcaaccccgacggctccctgctgttccgagtaaccatcaacggagtgaccggctggcggctgtgcgaacgcattctggcgtaattctagaaaaaaaaaaaaaaaaaaaaaaaaaaaaaa

SEQ ID NO: 35 - RNA, 24 nt, synthetic construct
  misc_feature 1..24: note = RNA5
  modified_base 1: mod_base = m7g
  misc_feature 1^2: note = triphosphate linkage
  source 1..24: mol_type = other RNA
ggaacggttacagcaacgctgctg

SEQ ID NO: 36 - RNA, 24 nt, synthetic construct
  misc_feature 1..24: note = RNA6
  modified_base 1: mod_base = m7g
  misc_feature 1^2: note = triphosphate linkage
  source 1..24: mol_type = other RNA
gaccgctttgctggaatcgaggaa

SEQ ID NO: 37 - RNA, 24 nt, synthetic construct
  misc_feature 1..24: note = RNA7
  modified_base 1: mod_base = m7g
  misc_feature 1^2: note = triphosphate linkage
  source 1..24: mol_type = other RNA
ggataggtgtctttgtcggttaca

SEQ ID NO: 38 - RNA, 24 nt, synthetic construct
  misc_feature 1..24: note = RNA8
  modified_base 1: mod_base = m7g
  misc_feature 1^2: note = triphosphate linkage
  source 1..24: mol_type = other RNA
ggatttgcggtgctttgctggaat

SEQ ID NO: 39 - DNA, 1338 bp, synthetic construct
  misc_feature 1..1338: note = mRNA coding Renilla luciferase
  source 1..1338: mol_type = other DNA
ggtttctactttgcccgcccacagatgtagttttctctgcgcgtgtgcgttttccctcctccccgccctcagggtccacggccaccatggcgtattaggggcagcagtgcctgcggcagcattggcctttgcagcggcggcagcagcaccaggctctgcagcggcaacccccagcggcttaagccatggcgcttctcacggcattcagcagcagcgttgctgtaaccgacaaagacaccttcgaattaagcacattcctcgattccagcaaagcaccgcaacatgaccgaaatgagcttcctgagcagcgaggtgttggtgggggacttgatgtcccccttcgaccagtcgggtttgggggctgaggcttccaaggtgtacgaccccgagcaacgcaaacgcatgatcactgggcctcagtggtgggctcgctgcaagcaaatgaacgtgctggactccttcatcaactactatgattccgagaagcacgccgagaacgccgtgatttttctgcatggtaacgctgcctccagctacctgtggaggcacgtcgtgcctcacatcgagcccgtggctagatgcatcatccctgatctgatcggaatgggtaagtccggcaagagcgggaatggctcatatcgcctcctggatcactacaagtacctcaccgcttggttcgagctgctgaaccttccaaagaaaatcatctttgtgggccacgactggggggcttgtctggcctttcactactcctacgagcaccaagacaagatcaaggccatcgtccatgctgagagtgtcgtggacgtgatcgagtcctgggacgagtggcctgacatcgaggaggatatcgccctgatcaagagcgaagagggcgagaaaatggtgcttgagaataacttcttcgtcgagaccatgctcccaagcaagatcatgcggaaactggagcctgaggagttcgctgcctacctggagccattcaaggagaagggcgaggttagacggcctaccctctcctggcctcgcgagatccctctcgttaagggaggcaagcccgacgtcgtccagattgtccgcaactacaacgcctaccttcgggccagcgacgatctgcctaagatgttcatcgagtccgaccctgggttcttttccaacgctattgtcgagggagctaagaagttccctaacaccgagttcgtgaaggtgaagggcctccacttcagccaggaggacgctccagatgaaatgggtaagtacatcaagagcttcgtggagcgcgtgctgaagaacgagcagtaattctaggcgaaaaaaaaaaaaaaaaaaaaaaaaaaaaaa

SEQ ID NO: 40 - DNA, 1276 bp, synthetic construct
  misc_feature 1..1276: note = IRES+NanoLuc DNA
  source 1..1276: mol_type = other DNA
cccggatcctaatacgactcactataggcgcatattaaggtgacgcgtaattcacgcgtcgagcatgcatctagggcggccaattccgcccctctcccccccccccctctccctcccccccccctaacgttactggccgaagccgcttggaataaggccggtgtgcgtttgtctatatgttattttccaccatattgccgtcttttggcaatgtgagggcccggaaacctggccctgtcttcttgacgagcattcctaggggtctttcccctctcgccaaaggaatgcaaggtctgttgaatgtcgtgaaggaagcagttcctctggaagcttcttgaagacaaacaacgtctgtagcgaccctttgcaggcagcggaaccccccacctggcgacaggtgcctctgcggccaaaagccacgtgtataagatacacctgcaaaggcggcacaaccccagtgccacgttgtgagttggatagttgtggaaagagtcaaatggctctcctcaagcgtattcaacaaggggctgaaggatgcccagaaggtaccccattgtatgggatctgatctggggcctcggtgcacatgctttacatgtgtttagtcgaggttaaaaaaacgtctaggccccccgaaccacggggacgtggttttcctttgaaaaacacgatgataagcttgccacaacccgggatcgccaccatggtcttcacactcgaagatttcgttggggactggcgacagacagccggctacaacctggaccaagtccttgaacagggaggtgtgtccagtttgtttcagaatctcggggtgtccgtaactccgatccaaaggattgtcctgagcggtgaaaatgggctgaagatcgacatccatgtcatcatcccgtatgaaggtctgagcggcgaccaaatgggccagatcgaaaaaatttttaaggtggtgtaccctgtggatgatcatcactttaaggtgatcctgcactatggcacactggtaatcgacggggttacgccgaacatgatcgactatttcggacggccgtatgaaggcatcgccgtgttcgacggcaaaaagatcactgtaacagggaccctgtggaacggcaacaaaattatcgacgagcgcctgatcaaccccgacggctccctgctgttccgagtaaccatcaacggagtgaccggctggcggctgtgcgaacgcattctggcgtaattctagagtcggggcggccggccgcttaaaaaaaaaaaaaaaaaaaaaaaaaaaaaa

SEQ ID NO: 41 - DNA, 4396 bp, synthetic construct
  misc_feature 1..4396: note = pIRES Vector + pNL1.1 TK Vector
  source 1..4396: mol_type = other DNA
ggcctaactggccggtacctgagtctaaatgagtcttcggacctcgcgggggccgcttaagcggtggttagggtttgtctgacgcggggggagggggaaggaacgaaacactctcattcggaggcggctcggggtttggtcttggtggccacgggcacgcagaagagcgccgcgatcctcttaagcacccccccgccctccgtggaggcgggggtttggtcggcgggtggtaactggcgggccgctgactcgggcgggtcgcgcgccccagagtgtgaccttttcggtctgctcgcagacccccgggcggcgccgccgcggcggcgacgggctcgctgggtcctaggctccatggggaccgtatacgtggacaggctctggagcatccgcacgactgcggtgatattaccggagaccttctgcgggacgagccgggtcacgcggctgacgcggagcgtccgttgggcgacaaacaccaggacggggcacaggtacactatcttgtcacccggaggcgcgagggactgcaggagcttcagggagtggcgcagctgcttcatccccgtggcccgttgctcgcgtttgctggcggtgtccccggaagaaatatatttgcatgtctttagttctatgatgacacaaaccccgcccagcgtcttgtcattggcgaattcgaacacgcagatgcagtcggggcggcgcggtcccaggtccacttcgcatattaaggtgacgcgtaattcacgcgtcgagcatgcatctagggcggccaattccgcccctctcccccccccccctctccctcccccccccctaacgttactggccgaagccgcttggaataaggccggtgtgcgtttgtctatatgttattttccaccatattgccgtcttttggcaatgtgagggcccggaaacctggccctgtcttcttgacgagcattcctaggggtctttcccctctcgccaaaggaatgcaaggtctgttgaatgtcgtgaaggaagcagttcctctggaagcttcttgaagacaaacaacgtctgtagcgaccctttgcaggcagcggaaccccccacctggcgacaggtgcctctgcggccaaaagccacgtgtataagatacacctgcaaaggcggcacaaccccagtgccacgttgtgagttggatagttgtggaaagagtcaaatggctctcctcaagcgtattcaacaaggggctgaaggatgcccagaaggtaccccattgtatgggatctgatctggggcctcggtgcacatgctttacatgtgtttagtcgaggttaaaaaaacgtctaggccccccgaaccacggggacgtggttttcctttgaaaaacacgatgataagcttgccacaacccgggatcgccaccatggtcttcacactcgaagatttcgttggggactggcgacagacagccggctacaacctggaccaagtccttgaacagggaggtgtgtccagtttgtttcagaatctcggggtgtccgtaactccgatccaaaggattgtcctgagcggtgaaaatgggctgaagatcgacatccatgtcatcatcccgtatgaaggtctgagcggcgaccaaatgggccagatcgaaaaaatttttaaggtggtgtaccctgtggatgatcatcactttaaggtgatcctgcactatggcacactggtaatcgacggggttacgccgaacatgatcgactatttcggacggccgtatgaaggcatcgccgtgttcgacggcaaaaagatcactgtaacagggaccctgtggaacggcaacaaaattatcgacgagcgcctgatcaaccccgacggctccctgctgttccgagtaaccatcaacggagtgaccggctggcggctgtgcgaacgcattctggcgtaattctagagtcggggcggccggccgcttcgagcagacatgataagatacattgatgagtttggacaaaccacaactagaatgcagtgaaaaaaatgctttatttgtgaaatttgtgatgctattgctttatttgtaaccattataagctgcaataaacaagttaacaacaacaattgcattcattttatgtttcaggttcagggggaggtgtgggaggttttttaaagcaagtaaaacctctacaaatgtggtaaaatcgataaggatccgtcgaccgatgcccttgagagccttcaacccagtcagctccttccggtgggcgcggggcatgactatcgtcgccgcacttatgactgtcttctttatcatgcaactcgtaggacaggtgccggcagcgctcttccgcttcctcgctcactgactcgctgcgctcggtcgttcggctgcggcgagcggtatcagctcactcaaaggcggtaatacggttatccacagaatcaggggataacgcaggaaagaacatgtgagcaaaaggccagcaaaaggccaggaaccgtaaaaaggccgcgttgctggcgtttttccataggctccgcccccctgacgagcatcacaaaaatcgacgctcaagtcagaggtggcgaaacccgacaggactataaagataccaggcgtttccccctggaagctccctcgtgcgctctcctgttccgaccctgccgcttaccggatacctgtccgcctttctcccttcgggaagcgtggcgctttctcatagctcacgctgtaggtatctcagttcggtgtaggtcgttcgctccaagctgggctgtgtgcacgaaccccccgttcagcccgaccgctgcgccttatccggtaactatcgtcttgagtccaacccggtaagacacgacttatcgccactggcagcagccactggtaacaggattagcagagcgaggtatgtaggcggtgctacagagttcttgaagtggtggcctaactacggctacactagaagaacagtatttggtatctgcgctctgctgaagccagttaccttcggaaaaagagttggtagctcttgatccggcaaacaaaccaccgctggtagcggtggtttttttgtttgcaagcagcagattacgcgcagaaaaaaaggatctcaagaagatcctttgatcttttctacggggtctgacgctcagtggaacgaaaactcacgttaagggattttggtcatgagattatcaaaaaggatcttcacctagatccttttaaattaaaaatgaagttttaaatcaatctaaagtatatatgagtaaacttggtctgacagcggccgcaaatgctaaaccactgcagtggttaccagtgcttgatcagtgaggcaccgatctcagcgatctgcctatttcgttcgtccatagtggcctgactccccgtcgtgtagatcactacgattcgtgagggcttaccatcaggccccagcgcagcaatgatgccgcgagagccgcgttcaccggcccccgatttgtcagcaatgaaccagccagcagggagggccgagcgaagaagtggtcctgctactttgtccgcctccatccagtctatgagctgctgtcgtgatgctagagtaagaagttcgccagtgagtagtttccgaagagttgtggccattgctactggcatcgtggtatcacgctcgtcgttcggtatggcttcgttcaactctggttcccagcggtcaagccgggtcacatgatcacccatattatgaagaaatgcagtcagctccttagggcctccgatcgttgtcagaagtaagttggccgcggtgttgtcgctcatggtaatggcagcactacacaattctcttaccgtcatgccatccgtaagatgcttttccgtgaccggcgagtactcaaccaagtcgttttgtgagtagtgtatacggcgaccaagctgctcttgcccggcgtctatacgggacaacaccgcgccacatagcagtactttgaaagtgctcatcatcgggaatcgttcttcggggcggaaagactcaaggatcttgccgctattgagatccagttcgatatagcccactcttgcacccagttgatcttcagcatcttttactttcaccagcgtttcggggtgtgcaaaaacaggcaagcaaaatgccgcaaagaagggaatgagtgcgacacgaaaatgttggatgctcatactcgtcctttttcaatattattgaagcatttatcagggttactagtacgtctctcaaggataagtaagtaatattaaggtacgggaggtattggacaggccgcaataaaatatctttattttcattacatctgtgtgttggttttttgtgtgaatcgatagtactaacatacgctctccatcaaaacaaaacgaaacaaaacaaactagcaaaataggctgtccccagtgcaagtgcaggtgccagaacatttctct

SEQ ID NO: 42 - DNA, 48 bp, synthetic construct
  misc_feature 1..48: note = synthetic oligo DNA
  source 1..48: mol_type = other DNA
cccggatcctaatacgactcactataggcgcatattaaggtgacgcgt

SEQ ID NO: 43 - DNA, 51 bp, synthetic construct; identical to SEQ ID NO: 26
  misc_feature 1..51: note = synthetic oligo DNA 2
  source 1..51: mol_type = other DNA

SEQ ID NO: 44 - RNA, 54 nt, synthetic construct; identical to SEQ ID NO: 33
  misc_feature 1..54: note = 54-nt flagment A
  source 1..54: mol_type = other RNA

SEQ ID NO: 45 - RNA, 54 nt, synthetic construct; identical to SEQ ID NO: 33
  misc_feature 1..54: note = 54-nt flagment B
  misc_feature 44^45: note = Two adenosines(A)-(A) are linked by a branching linker. 5'pG islinked to the branched chain that branches off from the mainchain.
  source 1..54: mol_type = other RNA

SEQ ID NO: 46 - RNA, 54 nt, synthetic construct; identical to SEQ ID NO: 33
  misc_feature 1..54: note = 54-nt flagment C
  misc_feature 44^45
  source 1..54: mol_type = other RNA

SEQ ID NO: 47 - RNA, 54 nt, synthetic construct; identical to SEQ ID NO: 33
  misc_feature 1..54: note = 54-nt flagment D
  misc_feature 14^15: note = The guanosine(G) and the uridine(U) are linked by a branchinglinker. 5'G is linked to the branched chain that branches offfrom the main chain.
  source 1..54: mol_type = other RNA

SEQ ID NO: 48 - RNA, 54 nt, synthetic construct; identical to SEQ ID NO: 33
  misc_feature 1..54: note = 54-nt flagment E
  misc_feature 14^15: note = The guanosine(G) and the uridine(U) are linked by a branchinglinker. 5'm7G-ppp-G is linked to the branched chain that branchesoff from the main chain.("5'm7G" indicates CAP structure).
  source 1..54: mol_type = other RNA

SEQ ID NO: 49 - RNA, 550 nt, synthetic construct
  misc_feature 1..550: note = 550-nt flagment (IVT synthesized)
  source 1..550: mol_type = other RNA
ggtcttcacactcgaagatttcgttggggactggcgacagacagccggctacaacctggaccaagtccttgaacagggaggtgtgtccagtttgtttcagaatctcggggtgtccgtaactccgatccaaaggattgtcctgagcggtgaaaatgggctgaagatcgacatccatgtcatcatcccgtatgaaggtctgagcggcgaccaaatgggccagatcgaaaaaatttttaaggtggtgtaccctgtggatgatcatcactttaaggtgatcctgcactatggcacactggtaatcgacggggttacgccgaacatgatcgactatttcggacggccgtatgaaggcatcgccgtgttcgacggcaaaaagatcactgtaacagggaccctgtggaacggcaacaaaattatcgacgagcgcctgatcaaccccgacggctccctgctgttccgagtaaccatcaacggagtgaccggctggcggctgtgcgaacgcattctggcgtaattctagaaaaaaaaaaaaaaaaaaaaaaaaaaaaaa

SEQ ID NO: 50 - RNA, 54 nt, synthetic construct; identical to SEQ ID NO: 33
  misc_feature 1..54: note = 54-nt flagment (n=6)
  misc_feature 44^45: note = Two adenosines(A)-(A) are linked by a branching linker.5'm7G-ppp-GmGmAGCGA is linked to the branched chain that branchesoff from the main chain.("5'm7G" indicates CAP structure. "Gm"indicates 2'OMe guanosine)
  source 1..54: mol_type = other RNA

SEQ ID NO: 51 - RNA, 54 nt, synthetic construct; identical to SEQ ID NO: 33
  misc_feature 1..54: note = 54-nt flagment (n=12)
  misc_feature 44^45: note = Two adenosines(A)-(A) are linked by a branching linker.5'm7G-ppp-GmGmAGCGAUAAA is linked to the branched chain thatbranches off from the main chain.("5'm7G" indicates CAPstructure. "Gm" indicates 2'OMe guanosine)
  source 1..54: mol_type = other RNA

SEQ ID NO: 52 - RNA, 24 nt, artificial sequence
  source 1..24: mol_type = mRNA
  misc_feature 1: note = 5' m7g
  misc_feature 1^2: note = triphosphate linkage
ggaacggttacagcaacgctgctg

SEQ ID NO: 53 - RNA, 24 nt, artificial sequence
  source 1..24: mol_type = mRNA
  misc_feature 1: note = 5' m7g
  misc_feature 1^2: note = triphosphate linkage
gaccgctttgctggaatcgaggaa

SEQ ID NO: 54 - RNA, 24 nt, artificial sequence
  source 1..24: mol_type = mRNA
  misc_feature 1: note = 5' m7g
  misc_feature 1^2: note = triphosphate linkage
ggataggtgtctttgtcggttaca

SEQ ID NO: 55 - RNA, 24 nt, artificial sequence
  source 1..24: mol_type = mRNA
  misc_feature 1: note = 5' m7g
  misc_feature 1^2: note = triphosphate linkage
ggatttgcggtgctttgctggaat

SEQ ID NO: 56 - RNA, 51 nt, artificial sequence; identical to SEQ ID NO: 7
  source 1..51: mol_type = mRNA
  misc_feature 1: note = 5' m7g
  misc_feature 1^2: note = triphosphate linkage

SEQ ID NO: 57 - RNA, 51 nt, artificial sequence; identical to SEQ ID NO: 7
  source 1..51: mol_type = mRNA
  misc_feature 1: note = 5' m7g
  misc_feature 1^2: note = triphosphate linkage
  misc_feature 2^3: note = 2'-methyl guanosine(Gm)

SEQ ID NO: 58 - RNA, 51 nt, artificial sequence; identical to SEQ ID NO: 7
  source 1..51: mol_type = mRNA
  misc_feature 1: note = 5' m7g
  misc_feature 1^2: note = triphosphate linkage
  misc_feature 2..4: note = LNA
  misc_feature 19..21: note = LNA

SEQ ID NO: 59 - RNA, 26 nt, artificial sequence
  source 1..26: mol_type = mRNA
  misc_feature 1: note = 5' m7g
  misc_feature 1^2: note = triphosphate linkage
ggagcggcgtcaccttaatatgcgcc

SEQ ID NO: 60 - RNA, 26 nt, artificial sequence
  source 1..26: mol_type = mRNA
  misc_feature 1: note = 5' m7g
  misc_feature 1^2: note = triphosphate linkage
  misc_feature 17..26: note = LNA
ggagcggcgtcaccttaatatgcgcc

SEQ ID NO: 61 - RNA, 26 nt, artificial sequence
  source 1..26: mol_type = mRNA
  misc_feature 1: note = 5' m7g
  misc_feature 1^2: note = triphosphate linkage
  misc_feature 22..26: note = LNA
ggagcggcgtcaccttaatatgcgcc

SEQ ID NO: 62 - RNA, 26 nt, artificial sequence
  source 1..26: mol_type = mRNA
  misc_feature 1: note = 5' m7g
  misc_feature 1^2: note = triphosphate linkage
  misc_feature 8: note = LNA
  misc_feature 10: note = LNA
  misc_feature 12: note = LNA
  misc_feature 14: note = LNA
  misc_feature 16: note = LNA
  misc_feature 18: note = LNA
  misc_feature 20: note = LNA
  misc_feature 22: note = LNA
  misc_feature 24: note = LNA
  misc_feature 26: note = LNA
ggagcggcgtcaccttaatatgcgcc

SEQ ID NO: 63 - RNA, 26 nt, artificial sequence
  source 1..26: mol_type = mRNA
  misc_feature 1: note = 5' m7g
  misc_feature 1^2: note = triphosphate linkage
  misc_feature 16: note = LNA
  misc_feature 18: note = LNA
  misc_feature 20: note = LNA
  misc_feature 22: note = LNA
  misc_feature 24: note = LNA
  misc_feature 26: note = LNA
ggagcggcgtcaccttaatatgcgcc

SEQ ID NO: 64 - RNA, 26 nt, artificial sequence
  source 1..26: mol_type = mRNA
  misc_feature 1: note = 5' m7g
  misc_feature 1^2: note = triphosphate linkage
  misc_feature 9: note = LNA
  misc_feature 12: note = LNA
  misc_feature 15: note = LNA
  misc_feature 18: note = LNA
  misc_feature 21: note = LNA
  misc_feature 24: note = LNA
ggagcggcgtcaccttaatatgcgcc